European Patent Application EP 4 660 320 A1, published December 10, 2025. Title: Method for detecting target RNA and kit therefore. Applicant: ＴＯＰＰＡＮホールディングス株式会社. Application WO. The sequence listing filed with the application follows.

SEQUENCE LISTING (11 sequences)

SEQ ID NO: 1 - RNA, 140 nt, synthetic construct
  source 1..140: mol_type = other RNA
gccaggatgtttcctaacgcgccctacctgcccagctgcctcgagagccagcccgctattcgcaatcagggttacagcacggtcaccttcgacgggacgcccagctacggtcacacgccctcgcaccatgcggcgcagtt

SEQ ID NO: 2 - DNA, 18 bp, synthetic construct
  source 1..18: mol_type = other DNA
aactgcgccgcatggtgc

SEQ ID NO: 3 - DNA, 15 bp, synthetic construct
  source 1..15: mol_type = other DNA
aactgcgccgcatgg

SEQ ID NO: 4 - DNA, 20 bp, synthetic construct
  source 1..20: mol_type = other DNA
cgcaatcagggttacagcac

SEQ ID NO: 5 - DNA, 18 bp, synthetic construct
  source 1..18: mol_type = other DNA
  modified_base 1: mod_base = OTHER; note = modified with VIC
  modified_base 18: mod_base = OTHER; note = Modified with MGB
cgtcccgtcgaaggtgac

SEQ ID NO: 6 - DNA, 25 bp, synthetic construct
  source 1..25: mol_type = other DNA
cgcgccgagggttacagcacggtca

SEQ ID NO: 7 - DNA, 33 bp, synthetic construct
  source 1..33: mol_type = other DNA
cctcgagagccagcccgctattcgcaatcagga

SEQ ID NO: 8 - DNA, 35 bp, synthetic construct
  source 1..35: mol_type = other DNA
  modified_base 1: mod_base = OTHER; note = Modified with Alexa488
  modified_base 5: mod_base = OTHER; note = Modified with BHQ1
ttcttagccggttttccggctgagacctcggcgcg

SEQ ID NO: 9 - DNA, 20 bp, synthetic construct
  source 1..20: mol_type = other DNA
cgcaatcagggttacagcac

SEQ ID NO: 10 - DNA, 18 bp, synthetic construct
  source 1..18: mol_type = other DNA
gtgcgagggcgtgtgacc

SEQ ID NO: 11 - DNA, 140 bp, synthetic construct
  source 1..140: mol_type = other DNA
aactgcgccgcatggtgcgagggcgtgtgaccgtagctgggcgtcccgtcgaaggtgaccgtgctgtaaccctgattgcgaatagcgggctggctctcgaggcagctgggcaggtagggcgcgttaggaaacatcctggc